European Patent Specification EP 3 369 816 B1, published March 13, 2024. Title: Composition stably containing single strand nucleic acid molecule suppressing expression of TGF-1. Applicant: BONAC CORPORATION TAKEUCHI, Hirofumi. Application EP 16859995.9. The sequence listing filed with the application follows.

SEQUENCE LISTING (2 sequences)

SEQ ID NO: 1 - RNA, 24 nt, Artificial Sequence
  nucleic acid molecule
agcagaguacacacagcauauacc

SEQ ID NO: 2 - RNA, 26 nt, Artificial Sequence
  nucleic acid molecule
gguauaugcuguguguacucugcuuc